European Patent Application EP 4 527 934 A1, published March 26, 2025. Title: GENE CARRIER BASED ON METAL NANO PARTICLE-NUCLEIC ACID CONJUGATE. Applicant: NESbiotechnology. Application KR 10-2022-0059957, filed May 17, 2022. The sequence listing filed with the application follows.

SEQUENCE LISTING (9 sequences)

SEQ ID NO: 1 - DNA, 5985 bp, synthetic construct
  source 1..5985: mol_type = other DNA
cttagggttaggcgttttgcgctgcttcgcgatgtacgggccagatatacgcgttgacattgattattgactagttattaatagtaatcaattacggggtcattagttcatagcccatatatggagttccgcgttacataacttacggtaaatggcccgcctggctgaccgcccaacgacccccgcccattgacgtcaataatgacgtatgttcccatagtaacgccaatagggactttccattgacgtcaatgggtggagtatttacggtaaactgcccacttggcagtacatcaagtgtatcatatgccaagtacgccccctattgacgtcaatgacggtaaatggcccgcctggcattatgcccagtacatgaccttatgggactttcctacttggcagtacatctacgtattagtcatcgctattaccatggtgatgcggttttggcagtacatcaatgggcgtggatagcggtttgactcacggggatttccaagtctccaccccattgacgtcaatgggagtttgttttggcaccaaaatcaacgggactttccaaaatgtcgtaacaactccgccccattgacgcaaatgggcggtaggcgtgtacggtgggaggtctatataagcagagctctctggctaactagagaacccactgcttactggcgccgccaccatggtgagcaagggcgaggagctgttcaccggggtggtgcccatcctggtcgagctggacggcgacgtaaacggccacaagttcagcgtgtccggcgagggcgagggcgatgccacctacggcaagctgaccctgaagttcatctgcaccaccggcaagctgcccgtgccctggcccaccctcgtgaccaccctgacctacggcgtgcagtgcttcagccgctaccccgaccacatgaagcagcacgacttcttcaagtccgccatgcccgaaggctacgtccaggagcgcaccatcttcttcaaggacgacggcaactacaagacccgcgccgaggtgaagttcgagggcgacaccctggtgaaccgcatcgagctgaagggcatcgacttcaaggaggacggcaacatcctggggcacaagctggagtacaactacaacagccacaacgtctatatcatggccgacaagcagaagaacggcatcaaggtgaacttcaagatccgccacaacatcgaggacggcagcgtgcagctcgccgaccactaccagcagaacacccccatcggcgacggccccgtgctgctgcccgacaaccactacctgagcacccagtccgccctgagcaaagaccccaacgagaagcgcgatcacatggtcctgctggagttcgtgaccgccgccgggatcactctcggcatggacgagctgtacaagtaacgactgtgccttctagttgccagccatctgttgtttgcccctcccccgtgccttccttgaccctggaaggtgccactcccactgtcctttcctaataaaatgaggaaattgcatcgcattgtctgagtaggtgtcattctattctggggggtggggtggggcaggacagcaagggggaggattgggaagacaatagcaggcatgctggggatgcggtgggctctatggcttctgaggcggaaagaaccagctggggctctagggggtatccccacgcgccctgtagcggcgcattaagcgcggcgggtgtggtggttacgcgcagcgtgaccgctacacttgccagcgccctagcgcccgctcctttcgctttcttcccttcctttctcgccacgttcgccggctttccccgtcaagctctaaatcgggggctccctttagggttccgatttagtgctttacggcacctcgaccccaaaaaacttgattagggtgatggttcacgtagtgggccatcgccctgatagacggtttttcgccctttgacgttggagtccacgttctttaatagtggactcttgttccaaactggaacaacactcaaccctatctcggtctattcttttgatttataagggattttgccgatttcggcctattggttaaaaaatgagctgatttaacaaaaatttaacgcgaattaattctgtggaatgtgtgtcagttagggtgtggaaagtccccaggctccccagcaggcagaagtatgcaaagcatgcatctcaattagtcagcaaccaggtgtggaaagtccccaggctccccagcaggcagaagtatgcaaagcatgcatctcaattagtcagcaaccatagtcccgcccctaactccgcccatcccgcccctaactccgcccagttccgcccattctccgccccatggctgactaattttttttatttatgcagaggccgaggccgcctctgcctctgagctattccagaagtagtgaggaggcttttttggaggcctaggcttttgcaaaaagctcccgggagcttgtatatccattttcggatctgatcaagagacaggatgaggatcgtttcgcatgattgaacaagatggattgcacgcaggttctccggccgcttgggtggagaggctattcggctatgactgggcacaacagacaatcggctgctctgatgccgccgtgttccggctgtcagcgcaggggcgcccggttctttttgtcaagaccgacctgtccggtgccctgaatgaactgcaggacgaggcagcgcggctatcgtggctggccacgacgggcgttccttgcgcagctgtgctcgacgttgtcactgaagcgggaagggactggctgctattgggcgaagtgccggggcaggatctcctgtcatctcaccttgctcctgccgagaaagtatccatcatggctgatgcaatgcggcggctgcatacgcttgatccggctacctgcccattcgaccaccaagcgaaacatcgcatcgagcgagcacgtactcggatggaagccggtcttgtcgatcaggatgatctggacgaagagcatcaggggctcgcgccagccgaactgttcgccaggctcaaggcgcgcatgcccgacggcgaggatctcgtcgtgacccatggcgatgcctgcttgccgaatatcatggtggaaaatggccgcttttctggattcatcgactgtggccggctgggtgtggcggaccgctatcaggacatagcgttggctacccgtgatattgctgaagagcttggcggcgaatgggctgaccgcttcctcgtgctttacggtatcgccgctcccgattcgcagcgcatcgccttctatcgccttcttgacgagttcttctgagcgggactctggggttcgaaatgaccgaccaagcgacgcccaacctgccatcacgagatttcgattccaccgccgccttctatgaaaggttgggcttcggaatcgttttccgggacgccggctggatgatcctccagcgcggggatctcatgctggagttcttcgcccaccccaacttgtttattgcagcttataatggttacaaataaagcaatagcatcacaaatttcacaaataaagcatttttttcactgcattctagttgtggtttgtccaaactcatcaatgtatcttatcatgtctgtataccgtcgacctctagctagagcttggcgtaatcatggtcatagctgtttcctgtgtgaaattgttatccgctcacaattccacacaacatacgagccggaagcataaagtgtaaagcctggggtgcctaatgagtgagctaactcacattaattgcgttgcgctcactgcccgctttccagtcgggaaacctgtcgtgccagctgcattaatgaatcggccaacgcgcggggagaggcggtttgcgtattgggcgctcttccgcttcctcgctcactgactcgctgcgctcggtcgttcggctgcggcgagcggtatcagctcactcaaaggcggtaatacggttatccacagaatcaggggataacgcaggaaagaacatgtgagcaaaaggccagcaaaaggccaggaaccgtaaaaaggccgcgttgctggcgtttttccataggctccgcccccctgacgagcatcacaaaaatcgacgctcaagtcagaggtggcgaaacccgacaggactataaagataccaggcgtttccccctggaagctccctcgtgcgctctcctgttccgaccctgccgcttaccggatacctgtccgcctttctcccttcgggaagcgtggcgctttctcatagctcacgctgtaggtatctcagttcggtgtaggtcgttcgctccaagctgggctgtgtgcacgaaccccccgttcagcccgaccgctgcgccttatccggtaactatcgtcttgagtccaacccggtaagacacgacttatcgccactggcagcagccactggtaacaggattagcagagcgaggtatgtaggcggtgctacagagttcttgaagtggtggcctaactacggctacactagaagaacagtatttggtatctgcgctctgctgaagccagttaccttcggaaaaagagttggtagctcttgatccggcaaacaaaccaccgctggtagcggtttttttgtttgcaagcagcagattacgcgcagaaaaaaaggatctcaagaagatcctttgatcttttctacggggtctgacgctcagtggaacgaaaactcacgttaagggattttggtcatgagattatcaaaaaggatcttcacctagatccttttaaattaaaaatgaagttttaaatcaatctaaagtatatatgagtaaacttggtctgacagttaccaatgcttaatcagtgaggcacctatctcagcgatctgtctatttcgttcatccatagttgcctgactccccgtcgtgtagataactacgatacgggagggcttaccatctggccccagtgctgcaatgataccgcgagacccacgctcaccggctccagatttatcagcaataaaccagccagccggaagggccgagcgcagaagtggtcctgcaactttatccgcctccatccagtctattaattgttgccgggaagctagagtaagtagttcgccagttaatagtttgcgcaacgttgttgccattgctacaggcatcgtggtgtcacgctcgtcgtttggtatggcttcattcagctccggttcccaacgatcaaggcgagttacatgatcccccatgttgtgcaaaaaagcggttagctccttcggtcctccgatcgttgtcagaagtaagttggccgcagtgttatcactcatggttatggcagcactgcataattctcttactgtcatgccatccgtaagatgcttttctgtgactggtgagtactcaaccaagtcattctgagaatagtgtatgcggcgaccgagttgctcttgcccggcgtcaatacgggataataccgcgccacatagcagaactttaaaagtgctcatcattggaaaacgttcttcggggcgaaaactctcaaggatcttaccgctgttgagatccagttcgatgtaacccactcgtgcacccaactgatcttcagcatcttttactttcaccagcgtttctgggtgagcaaaaacaggaaggcaaaatgccgcaaaaaagggaataagggcgacacggaaatgttgaatactcatactcttcctttttcaatattattgaagcatttatcagggttattgtctcatgagcggatacatatttgaatgtatttagaaaaataaacaaataggggttccgcgcacatttccccgaaaagtgccacctgacgtcgacggatcgggagatctcccgatcccctatggtgcactctcagtacaatctgctctgatgccgcatagttaagccagtatctgctccctgcttgtgtgttggaggtcgctgagtagtgcgcgagcaaaatttaagctacaacaaggcaaggcttgaccgacaattgcatgaagaatctg

SEQ ID NO: 2 - DNA, 1688 bp, synthetic construct
  source 1..1688: mol_type = other DNA
cttagggttaggcgttttgcgctgcttcgcgatgtacgggccagatatacgcgttgacattgattattgactagttattaatagtaatcaattacggggtcattagttcatagcccatatatggagttccgcgttacataacttacggtaaatggcccgcctggctgaccgcccaacgacccccgcccattgacgtcaataatgacgtatgttcccatagtaacgccaatagggactttccattgacgtcaatgggtggagtatttacggtaaactgcccacttggcagtacatcaagtgtatcatatgccaagtacgccccctattgacgtcaatgacggtaaatggcccgcctggcattatgcccagtacatgaccttatgggactttcctacttggcagtacatctacgtattagtcatcgctattaccatggtgatgcggttttggcagtacatcaatgggcgtggatagcggtttgactcacggggatttccaagtctccaccccattgacgtcaatgggagtttgttttggcaccaaaatcaacgggactttccaaaatgtcgtaacaactccgccccattgacgcaaatgggcggtaggcgtgtacggtgggaggtctatataagcagagctctctggctaactagagaacccactgcttactggcgccgccaccatggtgagcaagggcgaggagctgttcaccggggtggtgcccatcctggtcgagctggacggcgacgtaaacggccacaagttcagcgtgtccggcgagggcgagggcgatgccacctacggcaagctgaccctgaagttcatctgcaccaccggcaagctgcccgtgccctggcccaccctcgtgaccaccctgacctacggcgtgcagtgcttcagccgctaccccgaccacatgaagcagcacgacttcttcaagtccgccatgcccgaaggctacgtccaggagcgcaccatcttcttcaaggacgacggcaactacaagacccgcgccgaggtgaagttcgagggcgacaccctggtgaaccgcatcgagctgaagggcatcgacttcaaggaggacggcaacatcctggggcacaagctggagtacaactacaacagccacaacgtctatatcatggccgacaagcagaagaacggcatcaaggtgaacttcaagatccgccacaacatcgaggacggcagcgtgcagctcgccgaccactaccagcagaacacccccatcggcgacggccccgtgctgctgcccgacaaccactacctgagcacccagtccgccctgagcaaagaccccaacgagaagcgcgatcacatggtcctgctggagttcgtgaccgccgccgggatcactctcggcatggacgagctgtacaagtaacgactgtgccttctagttgccagccatctgttgtttgcccctcccccgtgccttccttgaccctggaaggtgccactcccactgtcctttcctaataaaatgaggaaattgcatcgcattgtctgagtaggtgtcattctattctggggggtggggtggggcaggacagcaagggggaggattgggaagacaatagcaggcatgctggggatgcggtgggctctatggcttctgaggcggaaagaaccagctggggctctagggggtatccccacgcgccctgtag

SEQ ID NO: 3 - DNA, 490 bp, synthetic construct
  source 1..490: mol_type = other DNA
gtgatgcggttttggcagtacatcaatgggcgtggatagcggtttgactcacggggatttccaagtctccaccccattgacgtcaatgggagtttgttttggcaccaaaatcaacgggactttccaaaatgtcgtaacaactccgccccattgacgcaaatgggcggtaggcgtgtacggtgggaggtctatataagcagagctctctggctaactagagaacccactgcttactggcgccgccaccatgaggcccgacaaaccaagaccatacctcccacggccaaggcccccgcgccctgttcgggactacaaggacgacgatgacaagtaacgactgtgccttctagttgccagccatctgttgtttgcccctcccccgtgccttccttgaccctggaaggtgccactcccactgtcctttcctaataaaatgaggaaattgcatcgcattgtctgagtaggtgtcattctattctggggggtgggg

SEQ ID NO: 4 - DNA, 469 bp, synthetic construct
  source 1..469: mol_type = other DNA
gtgatgcggttttggcagtacatcaatgggcgtggatagcggtttgactcacggggatttccaagtctccaccccattgacgtcaatgggagtttgttttggcaccaaaatcaacgggactttccaaaatgtcgtaacaactccgccccattgacgcaaatgggcggtaggcgtgtacggtgggaggtctatataagcagagctctctggctaactagagaacccactgcttactggcgccgccaccatgggctggcaaaatagcatccgccacaacctcagcctcgactacaaggacgacgatgacaagtaacgactgtgccttctagttgccagccatctgttgtttgcccctcccccgtgccttccttgaccctggaaggtgccactcccactgtcctttcctaataaaatgaggaaattgcatcgcattgtctgagtaggtgtcattctattctggggggtgggg

SEQ ID NO: 5 - DNA, 2617 bp, synthetic construct
  source 1..2617: mol_type = other DNA
cttagggttaggcgttttgcgctgcttcgcgatgtacgggccagatatacgcgttgacattgattattgactagttattaatagtaatcaattacggggtcattagttcatagcccatatatggagttccgcgttacataacttacggtaaatggcccgcctggctgaccgcccaacgacccccgcccattgacgtcaataatgacgtatgttcccatagtaacgccaatagggactttccattgacgtcaatgggtggagtatttacggtaaactgcccacttggcagtacatcaagtgtatcatatgccaagtacgccccctattgacgtcaatgacggtaaatggcccgcctggcattatgcccagtacatgaccttatgggactttcctacttggcagtacatctacgtattagtcatcgctattaccatggtgatgcggttttggcagtacatcaatgggcgtggatagcggtttgactcacggggatttccaagtctccaccccattgacgtcaatgggagtttgttttggcaccaaaatcaacgggactttccaaaatgtcgtaacaactccgccccattgacgcaaatgggcggtaggcgtgtacggtgggaggtctatataagcagagctctctggctaactagagaacccactgcttactggcgccgccaccatggaagacgccaaaaacataaagaaaggcccggcgccattctatccgctggaagatggaaccgctggagagcaactgcataaggctatgaagagatacgccctggttcctggaacaattgcttttacagatgcacatatcgaggtggacatcacttacgctgagtacttcgaaatgtccgttcggttggcagaagctatgaaacgatatgggctgaatacaaatcacagaatcgtcgtatgcagtgaaaactctcttcaattctttatgccggtgttgggcgcgttatttatcggagttgcagttgcgcccgcgaacgacatttataatgaacgtgaattgctcaacagtatgggcatttcgcagcctaccgtggtgttcgtttccaaaaaggggttgcaaaaaattttgaacgtgcaaaaaaagctcccaatcatccaaaaaattattatcatggattctaaaacggattaccagggatttcagtcgatgtacacgttcgtcacatctcatctacctcccggttttaatgaatacgattttgtgccagagtccttcgatagggacaagacaattgcactgatcatgaactcctctggatctactggtctgcctaaaggtgtcgctctgcctcatagaactgcctgcgtgagattctcgcatgccagagatcctatttttggcaatcaaatcattccggatactgcgattttaagtgttgttccattccatcacggttttggaatgtttactacactcggatatttgatatgtggatttcgagtcgtcttaatgtatagatttgaagaagagctgtttctgaggagccttcaggattacaagattcaaagtgcgctgctggtgccaaccctattctccttcttcgccaaaagcactctgattgacaaatacgatttatctaatttacacgaaattgcttctggtggcgctcccctctctaaggaagtcggggaagcggttgccaagaggttccatctgccaggtatcaggcaaggatatgggctcactgagactacatcagctattctgattacacccgagggggatgataaaccgggcgcggtcggtaaagttgttccattttttgaagcgaaggttgtggatctggataccgggaaaacgctgggcgttaatcaaagaggcgaactgtgtgtgagaggtcctatgattatgtccggttatgtaaacaatccggaagcgaccaacgccttgattgacaaggatggatggctacattctggagacatagcttactgggacgaagacgaacacttcttcatcgttgaccgcctgaagtctctgattaagtacaaaggctatcaggtggctcccgctgaattggaatccatcttgctccaacaccccaacatcttcgacgcaggtgtcgcaggtcttcccgacgatgacgccggtgaacttcccgccgccgttgttgttttggagcacggaaagacgatgacggaaaaagagatcgtggattacgtcgccagtcaagtaacaaccgcgaaaaagttgcgcggaggagttgtgtttgtggacgaagtaccgaaaggtcttaccggaaaactcgacgcaagaaaaatcagagagatcctcataaaggccaagaagggcggaaagatcgccgtgtaacgactgtgccttctagttgccagccatctgttgtttgcccctcccccgtgccttccttgaccctggaaggtgccactcccactgtcctttcctaataaaatgaggaaattgcatcgcattgtctgagtaggtgtcattctattctggggggtggggtggggacagcaagggggaggattgggaagacaatagcaggcatgctggggatgcggtgggctctatggcttctgaggcggaaagaaccagctggggctctagggggtatccccacgcgccctgtag

SEQ ID NO: 6 - DNA, 20 bp, synthetic construct
  source 1..20: mol_type = other DNA
cttagggttaggcgttttgc

SEQ ID NO: 7 - DNA, 21 bp, synthetic construct
  source 1..21: mol_type = other DNA
ctacagggcgcgtggggatac

SEQ ID NO: 8 - DNA, 19 bp, synthetic construct
  source 1..19: mol_type = other DNA
gtgatgcggttttggcagt

SEQ ID NO: 9 - DNA, 23 bp, synthetic construct
  source 1..23: mol_type = other DNA
ccccaccccccagaatagaatga